European Patent Application EP 4 400 594 A1, published July 17, 2024. Title: 改进的引导编辑系统. Applicant: 上海蓝十字医学科学研究所. Application CN. The sequence listing filed with the application follows.

SEQUENCE LISTING (19 sequences)

SEQ ID NO: 1 - protein, 1368 aa, S. pyogenes [sequence omitted]

SEQ ID NO: 2 - protein, 1368 aa, synthetic construct
MDKKYSIGLDIGTNSVGWAVITDEYKVPSKKFKVLGNTDRHSIKKNLIGALLFDSGETAEATRLKRTARRRYTRRKNRICYLQEIFSNEMAKVDDSFFHRLEESFLVEEDKKHERHPIFGNIVDEVAYHEKYPTIYHLRKKLVDSTDKADLRLIYLALAHMIKFRGHFLIEGDLNPDNSDVDKLFIQLVQTYNQLFEENPINASGVDAKAILSARLSKSRRLENLIAQLPGEKKNGLFGNLIALSLGLTPNFKSNFDLAEDAKLQLSKDTYDDDLDNLLAQIGDQYADLFLAAKNLSDAILLSDILRVNTEITKAPLSASMIKRYDEHHQDLTLLKALVRQQLPEKYKEIFFDQSKNGYAGYIDGGASQEEFYKFIKPILEKMDGTEELLVKLNREDLLRKQRTFDNGSIPHQIHLGELHAILRRQEDFYPFLKDNREKIEKILTFRIPYYVGPLARGNSRFAWMTRKSEETITPWNFEEVVDKGASAQSFIERMTNFDKNLPNEKVLPKHSLLYEYFTVYNELTKVKYVTEGMRKPAFLSGEQKKAIVDLLFKTNRKVTVKQLKEDYFKKIECFDSVEISGVEDRFNASLGTYHDLLKIIKDKDFLDNEENEDILEDIVLTLTLFEDREMIEERLKTYAHLFDDKVMKQLKRRRYTGWGRLSRKLINGIRDKQSGKTILDFLKSDGFANRNFMQLIHDDSLTFKEDIQKAQVSGQGDSLHEHIANLAGSPAIKKGILQTVKVVDELVKVMGRHKPENIVIEMARENQTTQKGQKNSRERMKRIEEGIKELGSQILKEHPVENTQLQNEKLYLYYLQNGRDMYVDQELDINRLSDYDVDAIVPQSFLKDDSIDNKVLTRSDKNRGKSDNVPSEEVVKKMKNYWRQLLNAKLITQRKFDNLTKAERGGLSELDKAGFIKRQLVETRQITKHVAQILDSRMNTKYDENDKLIREVKVITLKSKLVSDFRKDFQFYKVREINNYHHAHDAYLNAVVGTALIKKYPKLESEFVYGDYKVYDVRKMIAKSEQEIGKATAKYFFYSNIMNFFKTEITLANGEIRKRPLIETNGETGEIVWDKGRDFATVRKVLSMPQVNIVKKTEVQTGGFSKESILPKRNSDKLIARKKDWDPKKYGGFDSPTVAYSVLVVAKVEKGKSKKLKSVKELLGITIMERSSFEKNPIDFLEAKGYKEVKKDLIIKLPKYSLFELENGRKRMLASAGELQKGNELALPSKYVNFLYLASHYEKLKGSPEDNEQKQLFVEQHKHYLDEIIEQISEFSKRVILADANLDKVLSAYNKHRDKPIREQAENIIHLFTLTNLGAPAAFKYFDTTIDRKRYTSTKEVLDATLIHQSITGLYETRIDLSQLGGD

SEQ ID NO: 3 - protein, 677 aa, Moloney Murine Leukemia Virus
TLNIEDEYRLHETSKEPDVSLGSTWLSDFPQAWAETGGMGLAVRQAPLIIPLKATSTPVSIKQYPMSQEARLGIKPHIQRLLDQGILVPCQSPWNTPLLPVKKPGTNDYRPVQDLREVNKRVEDIHPTVPNPYNLLSGLPPSHQWYTVLDLKDAFFCLRLHPTSQPLFAFEWRDPEMGISGQLTWTRLPQGFKNSPTLFNEALHRDLADFRIQHPDLILLQYVDDLLLAATSELDCQQGTRALLQTLGNLGYRASAKKAQICQKQVKYLGYLLKEGQRWLTEARKETVMGQPTPKTPRQLREFLGKAGFCRLFIPGFAEMAAPLYPLTKPGTLFNWGPDQQKAYQEIKQALLTAPALGLPDLTKPFELFVDEKQGYAKGVLTQKLGPWRRPVAYLSKKLDPVAAGWPPCLRMVAAIAVLTKDAGKLTMGQPLVILAPHAVEALVKQPPDRWLSNARMTHYQALLLDTDRVQFGPVVALNPATLLPLPEEGLQHNCLDILAEAHGTRPDLTDQPLPDADHTWYTDGSSLLQEGQRKAGAAVTTETEVIWAKALPAGTSAQRAELIALTQALKMAEGKKLNVYTDSRYAFATAHIHGEIYRRRGWLTSEGKEIKNKDEILALLKALFLPKRLSIIHCPGHQKGHSAEARGNRMADQAARKAAITETPDTSTLLIENSSP

SEQ ID NO: 4 - protein, 129 aa, synthetic construct
DQQKAYQEIKQALLTAPALGLPDLTKPFELFVDEKQGYAKGVLTQKLGPWRRPVAYLSKKLDPVAAGWPPCLRMVAAIAVLTKDAGKLTMGQPLVILAPHAVEALVKQPPDRWLSNARMTHYQALLLDT

SEQ ID NO: 5 - protein, 157 aa, synthetic construct
PDADHTWYTDGSSLLQEGQRKAGAAVTTETEVIWAKALPAGTSAQRAELIALTQALKMAEGKKLNVYTDSRYAFATAHIHGEIYRRRGWLTSEGKEIKNKDEILALLKALFLPKRLSIIHCPGHQKGHSAEARGNRMADQAARKAAITETPDTSTLL

SEQ ID NO: 6 - protein, 56 aa, synthetic construct
ATVVSGQKQDRQGGERRRSQLDRDQCAYCKEKGHWAKDCPKKPRGPRGPRPQTSLL

SEQ ID NO: 7 - protein, 125 aa, synthetic construct
TLDDQGGQGQEPPPEPRITLKVGGQPVTFLVDTGAQHSVLTQNPGPLSDKSAWVQGATGGKRYRWTTDRKVHLATGKVTHSFLHVPDCPYPLLGRDLLTKLKAQIHFEGSGAQVMGPMGQPLQVL

SEQ ID NO: 8 - protein, 407 aa, synthetic construct
ENSSPYTSEHFHYTVTDIKDLTKLGAIYDKTKKYWVYQGKPVMPDQFTFELLDFLHQLTHLSFSKMKALLERSHSPYYMLNRDRTLKNITETCKACAQVNASKSAVKQGTRVRGHRPGTHWEIDFTEIKPGLYGYKYLLVFIDTFSGWIEAFPTKKETAKVVTKKLLEEIFPRFGMPQVLGTDNGPAFVSKVSQTVADLLGIDWKLHCAYRPQSSGQVERMNRTIKETLTKLTLATGSRDWVLLLPLALYRARNTPGPHGLTPYEILYGAPPPLVNFPDPDMTRVTNSPSLQAHLQALYLVQHEVWRPLAAAYQEQLDRPVVPHPYRVGDTVWVRRHQTKNLEPRWKGPYTVLLTTPTALKVDGIAAWIHAAHVKAADPGGGPSSRLTWRVQRSQNPLKIRLTREAP

SEQ ID NO: 9 - protein, 677 aa, synthetic construct
TLNIEDEYRLHETSKEPDVSLGSTWLSDFPQAWAETGGMGLAVRQAPLIIPLKATSTPVSIKQYPMSQEARLGIKPHIQRLLDQGILVPCQSPWNTPLLPVKKPGTNDYRPVQDLREVNKRVEDIHPTVPNPYNLLSGLPPSHQWYTVLDLKDAYFCLRLHPTSQPLFAFEWRDPEMGISGQLTWTRLPQGFKNSPTLFNEALHRDLADFRIQHPDLILLQYVDDLLLAATSELDCQQGTRALLQTLGNLGYRASAKKAQICQKQVKYLGYLLKEGQRWLTEARKETVMGQPTPKTPRQLREFLGKAGFCRLFIPGFAEMAAPLYPLTKPGTLFNWGPDQQKAYQEIKQALLTAPALGLPDLTKPFELFVDEKQGYAKGVLTQKLGPWRRPVAYLSKKLDPVAAGWPPCLRMVAAIAVLTKDAGKLTMGQPLVILAPHAVEALVKQPPDRWLSNARMTHYQALLLDTDRVQFGPVVALNPATLLPLPEEGLQHNCLDILAEAHGTRPDLTDQPLPDADHTWYTDGSSLLQEGQRKAGAAVTTETEVIWAKALPAGTSAQRAELIALTQALKMAEGKKLNVYTDSRYAFATAHIHGEIYRRRGWLTSEGKEIKNKDEILALLKALFLPKRLSIIHCPGHQKGHSAEARGNRMADQAARKAAITETPDTSTLLIENSSP

SEQ ID NO: 10 - protein, 677 aa, synthetic construct
TLNIEDEYRLHETSKEPDVSLGSTWLSDFPQAWAETGGMGLAVRQAPLIIPLKATSTPVSIKQYPMSQEARLGIKPHIQRLLDQGILVPCQSPWNTPLLPVKKPGTNDYRPVQDLREVNKRVEDIHPTVPNPYNLLSGLPPSHQWYTVLDLKDAVFCLRLHPTSQPLFAFEWRDPEMGISGQLTWTRLPQGFKNSPTLFNEALHRDLADFRIQHPDLILLQYVDDLLLAATSELDCQQGTRALLQTLGNLGYRASAKKAQICQKQVKYLGYLLKEGQRWLTEARKETVMGQPTPKTPRQLREFLGKAGFCRLFIPGFAEMAAPLYPLTKPGTLFNWGPDQQKAYQEIKQALLTAPALGLPDLTKPFELFVDEKQGYAKGVLTQKLGPWRRPVAYLSKKLDPVAAGWPPCLRMVAAIAVLTKDAGKLTMGQPLVILAPHAVEALVKQPPDRWLSNARMTHYQALLLDTDRVQFGPVVALNPATLLPLPEEGLQHNCLDILAEAHGTRPDLTDQPLPDADHTWYTDGSSLLQEGQRKAGAAVTTETEVIWAKALPAGTSAQRAELIALTQALKMAEGKKLNVYTDSRYAFATAHIHGEIYRRRGWLTSEGKEIKNKDEILALLKALFLPKRLSIIHCPGHQKGHSAEARGNRMADQAARKAAITETPDTSTLLIENSSP

SEQ ID NO: 11 - protein, 677 aa, synthetic construct
TLNIEDEYRLHETSKEPDVSLGSTWLSDFPQAWAETGGMGLAVRQAPLIIPLKATSTPVSIKQYPMSQEARLGIKPHIQRLLDQGILVPCQSPWNTPLLPVKKPGTNDYRPVQDLREVNKRVEDIHPTVPNPYNLLSGLPPSHQWYTVLDLKDAFYCLRLHPTSQPLFAFEWRDPEMGISGQLTWTRLPQGFKNSPTLFNEALHRDLADFRIQHPDLILLQYVDDLLLAATSELDCQQGTRALLQTLGNLGYRASAKKAQICQKQVKYLGYLLKEGQRWLTEARKETVMGQPTPKTPRQLREFLGKAGFCRLFIPGFAEMAAPLYPLTKPGTLFNWGPDQQKAYQEIKQALLTAPALGLPDLTKPFELFVDEKQGYAKGVLTQKLGPWRRPVAYLSKKLDPVAAGWPPCLRMVAAIAVLTKDAGKLTMGQPLVILAPHAVEALVKQPPDRWLSNARMTHYQALLLDTDRVQFGPVVALNPATLLPLPEEGLQHNCLDILAEAHGTRPDLTDQPLPDADHTWYTDGSSLLQEGQRKAGAAVTTETEVIWAKALPAGTSAQRAELIALTQALKMAEGKKLNVYTDSRYAFATAHIHGEIYRRRGWLTSEGKEIKNKDEILALLKALFLPKRLSIIHCPGHQKGHSAEARGNRMADQAARKAAITETPDTSTLLIENSSP

SEQ ID NO: 12 - protein, 677 aa, synthetic construct
TLNIEDEYRLHETSKEPDVSLGSTWLSDFPQAWAETGGMGLAVRQAPLIIPLKATSTPVSIKQYPMSQEARLGIKPHIQRLLDQGILVPCQSPWNTPLLPVKKPGTNDYRPVQDLREVNKRVEDIHPTVPNPYNLLSGLPPSHQWYTVLDLKDAFFCLRLHPTSQPLFAFEWRDPEMGISGQLTWTRLPQGFKNSPTLFNEALHRDLADFRIQHPDLILLQYVDDLLLAATSELDCQQGTRALLQTLGNLGYRASAKKAQICQKQVKYLGYLLKEGQRWLTEARKETVMGQPTPKTPRQLREFLGKAGFCRLFIPGFAEMAAPLYPLTKPGTLFNWGPDQQKAYQEIKQALLTAPALGLPDLTKPFELFVDEKQGYAKGVLTQKLGPWRRPVAYLSKKLDPVAAGWPPCLRMVAAIAVLTKDAGKLTMGQPLVILAPHAVEALVKQPPDRWLSNARMTHYQALLLDTDRVQFGPVVALNPATLLPLPEEGLQHNCLDILAEAHGTRPDLTDQPLPDADHTWYTNGSSLLQEGQRKAGAAVTTETEVIWAKALPAGTSAQRAELIALTQALKMAEGKKLNVYTDSRYAFATAHIHGEIYRRRGWLTSEGKEIKNKDEILALLKALFLPKRLSIIHCPGHQKGHSAEARGNRMADQAARKAAITETPDTSTLLIENSSP

SEQ ID NO: 13 - protein, 677 aa, synthetic construct
TLNIEDEYRLHETSKEPDVSLGSTWLSDFPQAWAETGGMGLAVRQAPLIIPLKATSTPVSIKQYPMSQEARLGIKPHIQRLLDQGILVPCQSPWNTPLLPVKKPGTNDYRPVQDLREVNKRVEDIHPTVPNPYNLLSGLPPSHQWYTVLDLKDAYFCLRLHPTSQPLFAFEWRDPEMGISGQLTWTRLPQGFKNSPTLFCEALHRDLADFRIQHPDLILLQYVDDLLLAATSELDCQQGTRALLQTLGNLGYRASAKKAQICQKQVKYLGYLLKEGQRWLTEARKETVMGQPTPKTPRQLREFLGKAGFCRLFIPGFAEMAAPLYPLTKPGTLFNWGPDQQKAYQEIKQALLTAPALGLPDLTKPFELFVDEKQGYAKGVLTQKLGPWRRPVAYLSKKLDPVAAGWPPCLRMVAAIAVLTKDAGKLTMGQPLVILAPHAVEALVKQPPDRWLSNARMTHYQALLLDTDRVQFGPVVALNPATLLPLPEEGLQHNCLDILAEAHGTRPDLTDQPLPDADHTWYTDGSSLLQEGQRKAGAAVTTETEVIWAKALPAGTSAQRAELIALTQALKMAEGKKLNVYTDSRYAFATAHIHGEIYRRRGWLTSEGKEIKNKDEILALLKALFLPKRLSIIHCPGHQKGHSAEARGNRMADQAARKAAITETPDTSTLLIENSSP

SEQ ID NO: 14 - protein, 514 aa, synthetic construct
TLNIEDEYRLHETSKEPDVSLGSTWLSDFPQAWAETGGMGLAVRQAPLIIPLKATSTPVSIKQYPMSQEARLGIKPHIQRLLDQGILVPCQSPWNTPLLPVKKPGTNDYRPVQDLREVNKRVEDIHPTVPNPYNLLSGLPPSHQWYTVLDLKDAFFCLRLHPTSQPLFAFEWRDPEMGISGQLTWTRLPQGFKNSPTLFNEALHRDLADFRIQHPDLILLQYVDDLLLAATSELDCQQGTRALLQTLGNLGYRASAKKAQICQKQVKYLGYLLKEGQRWLTEARKETVMGQPTPKTPRQLREFLGKAGFCRLFIPGFAEMAAPLYPLTKPGTLFNWGPDQQKAYQEIKQALLTAPALGLPDLTKPFELFVDEKQGYAKGVLTQKLGPWRRPVAYLSKKLDPVAAGWPPCLRMVAAIAVLTKDAGKLTMGQPLVILAPHAVEALVKQPPDRWLSNARMTHYQALLLDTDRVQFGPVVALNPATLLPLPEEGLQHNCLDILAEAHGTRPDLTDQPL

SEQ ID NO: 15 - protein, 338 aa, synthetic construct
TLNIEDEYRLHETSKEPDVSLGSTWLSDFPQAWAETGGMGLAVRQAPLIIPLKATSTPVSIKQYPMSQEARLGIKPHIQRLLDQGILVPCQSPWNTPLLPVKKPGTNDYRPVQDLREVNKRVEDIHPTVPNPYNLLSGLPPSHQWYTVLDLKDAFFCLRLHPTSQPLFAFEWRDPEMGISGQLTWTRLPQGFKNSPTLFNEALHRDLADFRIQHPDLILLQYVDDLLLAATSELDCQQGTRALLQTLGNLGYRASAKKAQICQKQVKYLGYLLKEGQRWLTEARKETVMGQPTPKTPRQLREFLGKAGFCRLFIPGFAEMAAPLYPLTKPGTLFNWGP

SEQ ID NO: 16 - protein, 32 aa, synthetic construct
SGGSSGGSSGSETPGTSESATPESSGGSSGGS

SEQ ID NO: 17 - RNA, 75 nt, synthetic construct
  source 1..75: mol_type = other RNA
gtttagagctagaaatagcaagttaaaataaggctagtccgttatcaacttgaaaaagtggcaccgagtcggtgc

SEQ ID NO: 18 - protein, 2108 aa, synthetic construct
MPKKKRKVDKKYSIGLDIGTNSVGWAVITDEYKVPSKKFKVLGNTDRHSIKKNLIGALLFDSGETAEATRLKRTARRRYTRRKNRICYLQEIFSNEMAKVDDSFFHRLEESFLVEEDKKHERHPIFGNIVDEVAYHEKYPTIYHLRKKLVDSTDKADLRLIYLALAHMIKFRGHFLIEGDLNPDNSDVDKLFIQLVQTYNQLFEENPINASGVDAKAILSARLSKSRRLENLIAQLPGEKKNGLFGNLIALSLGLTPNFKSNFDLAEDAKLQLSKDTYDDDLDNLLAQIGDQYADLFLAAKNLSDAILLSDILRVNTEITKAPLSASMIKRYDEHHQDLTLLKALVRQQLPEKYKEIFFDQSKNGYAGYIDGGASQEEFYKFIKPILEKMDGTEELLVKLNREDLLRKQRTFDNGSIPHQIHLGELHAILRRQEDFYPFLKDNREKIEKILTFRIPYYVGPLARGNSRFAWMTRKSEETITPWNFEEVVDKGASAQSFIERMTNFDKNLPNEKVLPKHSLLYEYFTVYNELTKVKYVTEGMRKPAFLSGEQKKAIVDLLFKTNRKVTVKQLKEDYFKKIECFDSVEISGVEDRFNASLGTYHDLLKIIKDKDFLDNEENEDILEDIVLTLTLFEDREMIEERLKTYAHLFDDKVMKQLKRRRYTGWGRLSRKLINGIRDKQSGKTILDFLKSDGFANRNFMQLIHDDSLTFKEDIQKAQVSGQGDSLHEHIANLAGSPAIKKGILQTVKVVDELVKVMGRHKPENIVIEMARENQTTQKGQKNSRERMKRIEEGIKELGSQILKEHPVENTQLQNEKLYLYYLQNGRDMYVDQELDINRLSDYDVDAIVPQSFLKDDSIDNKVLTRSDKNRGKSDNVPSEEVVKKMKNYWRQLLNAKLITQRKFDNLTKAERGGLSELDKAGFIKRQLVETRQITKHVAQILDSRMNTKYDENDKLIREVKVITLKSKLVSDFRKDFQFYKVREINNYHHAHDAYLNAVVGTALIKKYPKLESEFVYGDYKVYDVRKMIAKSEQEIGKATAKYFFYSNIMNFFKTEITLANGEIRKRPLIETNGETGEIVWDKGRDFATVRKVLSMPQVNIVKKTEVQTGGFSKESILPKRNSDKLIARKKDWDPKKYGGFDSPTVAYSVLVVAKVEKGKSKKLKSVKELLGITIMERSSFEKNPIDFLEAKGYKEVKKDLIIKLPKYSLFELENGRKRMLASAGELQKGNELALPSKYVNFLYLASHYEKLKGSPEDNEQKQLFVEQHKHYLDEIIEQISEFSKRVILADANLDKVLSAYNKHRDKPIREQAENIIHLFTLTNLGAPAAFKYFDTTIDRKRYTSTKEVLDATLIHQSITGLYETRIDLSQLGGDEFPKKKRKVELSGGSSGGSSGSETPGTSESATPESSGGSSGGSRPTLNIEDEYRLHETSKEPDVSLGSTWLSDFPQAWAETGGMGLAVRQAPLIIPLKATSTPVSIKQYPMSQEARLGIKPHIQRLLDQGILVPCQSPWNTPLLPVKKPGTNDYRPVQDLREVNKRVEDIHPTVPNPYNLLSGLPPSHQWYTVLDLKDAFFCLRLHPTSQPLFAFEWRDPEMGISGQLTWTRLPQGFKNSPTLFNEALHRDLADFRIQHPDLILLQYVDDLLLAATSELDCQQGTRALLQTLGNLGYRASAKKAQICQKQVKYLGYLLKEGQRWLTEARKETVMGQPTPKTPRQLREFLGKAGFCRLFIPGFAEMAAPLYPLTKPGTLFNWGPDQQKAYQEIKQALLTAPALGLPDLTKPFELFVDEKQGYAKGVLTQKLGPWRRPVAYLSKKLDPVAAGWPPCLRMVAAIAVLTKDAGKLTMGQPLVILAPHAVEALVKQPPDRWLSNARMTHYQALLLDTDRVQFGPVVALNPATLLPLPEEGLQHNCLDILAEAHGTRPDLTDQPLPDADHTWYTDGSSLLQEGQRKAGAAVTTETEVIWAKALPAGTSAQRAELIALTQALKMAEGKKLNVYTDSRYAFATAHIHGEIYRRRGWLTSEGKEIKNKDEILALLKALFLPKRLSIIHCPGHQKGHSAEARGNRMADQAARKAAITETPDTSTLLIENSSPSGGSPKKKRKV

SEQ ID NO: 19 - protein, 2017 aa, synthetic construct
MPKKKRKVDKKYSIGLDIGTNSVGWAVITDEYKVPSKKFKVLGNTDRHSIKKNLIGALLFDSGETAEATRLKRTARRRYTRRKNRICYLQEIFSNEMAKVDDSFFHRLEESFLVEEDKKHERHPIFGNIVDEVAYHEKYPTIYHLRKKLVDSTDKADLRLIYLALAHMIKFRGHFLIEGDLNPDNSDVDKLFIQLVQTYNQLFEENPINASGVDAKAILSARLSKSRRLENLIAQLPGEKKNGLFGNLIALSLGLTPNFKSNFDLAEDAKLQLSKDTYDDDLDNLLAQIGDQYADLFLAAKNLSDAILLSDILRVNTEITKAPLSASMIKRYDEHHQDLTLLKALVRQQLPEKYKEIFFDQSKNGYAGYIDGGASQEEFYKFIKPILEKMDGTEELLVKLNREDLLRKQRTFDNGSIPHQIHLGELHAILRRQEDFYPFLKDNREKIEKILTFRIPYYVGPLARGNSRFAWMTRKSEETITPWNFEEVVDKGASAQSFIERMTNFDKNLPNEKVLPKHSLLYEYFTVYNELTKVKYVTEGMRKPAFLSGEQKKAIVDLLFKTNRKVTVKQLKEDYFKKIECFDSVEISGVEDRFNASLGTYHDLLKIIKDKDFLDNEENEDILEDIVLTLTLFEDREMIEERLKTYAHLFDDKVMKQLKRRRYTGWGRLSRKLINGIRDKQSGKTILDFLKSDGFANRNFMQLIHDDSLTFKEDIQKAQVSGQGDSLHEHIANLAGSPAIKKGILQTVKVVDELVKVMGRHKPENIVIEMARENQTTQKGQKNSRERMKRIEEGIKELGSQILKEHPVENTQLQNEKLYLYYLQNGRDMYVDQELDINRLSDYDVDAIVPQSFLKDDSIDNKVLTRSDKNRGKSDNVPSEEVVKKMKNYWRQLLNAKLITQRKFDNLTKAERGGLSELDKAGFIKRQLVETRQITKHVAQILDSRMNTKYDENDKLIREVKVITLKSKLVSDFRKDFQFYKVREINNYHHAHDAYLNAVVGTALIKKYPKLESEFVYGDYKVYDVRKMIAKSEQEIGKATAKYFFYSNIMNFFKTEITLANGEIRKRPLIETNGETGEIVWDKGRDFATVRKVLSMPQVNIVKKTEVQTGGFSKESILPKRNSDKLIARKKDWDPKKYGGFDSPTVAYSVLVVAKVEKGKSKKLKSVKELLGITIMERSSFEKNPIDFLEAKGYKEVKKDLIIKLPKYSLFELENGRKRMLASAGELQKGNELALPSKYVNFLYLASHYEKLKGSPEDNEQKQLFVEQHKHYLDEIIEQISEFSKRVILADANLDKVLSAYNKHRDKPIREQAENIIHLFTLTNLGAPAAFKYFDTTIDRKRYTSTKEVLDATLIHQSITGLYETRIDLSQLGGDEFSGSETPGTSESATPESATVVSGQKQDRQGGERRRSQLDRDQCAYCKEKGHWAKDCPKKPRGPRGPRPQTSLLPKKKRKVELSGGSSGGSSGSETPGTSESATPESSGGSSGGSRPTLNIEDEYRLHETSKEPDVSLGSTWLSDFPQAWAETGGMGLAVRQAPLIIPLKATSTPVSIKQYPMSQEARLGIKPHIQRLLDQGILVPCQSPWNTPLLPVKKPGTNDYRPVQDLREVNKRVEDIHPTVPNPYNLLSGLPPSHQWYTVLDLKDAFFCLRLHPTSQPLFAFEWRDPEMGISGQLTWTRLPQGFKNSPTLFNEALHRDLADFRIQHPDLILLQYVDDLLLAATSELDCQQGTRALLQTLGNLGYRASAKKAQICQKQVKYLGYLLKEGQRWLTEARKETVMGQPTPKTPRQLREFLGKAGFCRLFIPGFAEMAAPLYPLTKPGTLFNWGPDQQKAYQEIKQALLTAPALGLPDLTKPFELFVDEKQGYAKGVLTQKLGPWRRPVAYLSKKLDPVAAGWPPCLRMVAAIAVLTKDAGKLTMGQPLVILAPHAVEALVKQPPDRWLSNARMTHYQALLLDTDRVQFGPVVALNPATLLPLPEEGLQHNCLDILAEAHGTRPDLTDQPLSGGSPKKKRKV